European Patent Specification EP 3 476 948 B1, published January 21, 2026. Title: Verfahren und Vorrichtung zur Bestimmung der Blutgruppe einer Katze im AB-Blutgruppensystem. Applicant: LABOklin Labor für klinische Diagnostik GmbH & Co. KG. The sequence listing filed with the application follows.

SEQUENCE LISTING (44 sequences)

SEQ ID NO: 1 - DNA, 2147 bp, Felis catus
  Cytidin-Monophosphat-N-Acetylneuraminsäure-Hydroxylase (CMAH), CMAH-A Allel
atggagcaaagcattgaacagacgacggaggtcttgttgtgtctgtcacctggagaagctgctgacctgaaggaaggaatcaatttcttgagaaacaagaagaccggcaaagatttcattctgtacaagagcaagaatcgcgtgagggcgtgcaagaacgtgtgcaagcatcaaggaggcctgttcataaaagacatygaagatttagacggaaggtctgtcagatgcacaaagcacaactggaggttggatgtgagcaccatgaaatacgtcaatcccccaggcagcttctgtcaagacgaactagttgttgaaatggatgaagaaaatggacttttacttctagaactgaatcctcccaatccctgggattcagaacccagatctcctgaacatttggcttttggagaagtgcagatcacgtacctcacccacgcctgcatggacctcaagctgggagacaagaggatggtgtttgacccctggttaacgggtcctgcgttcgcccgaggctggtggctgctgcacgagcctccgtctgattggctggagaggctgtgccaggcagacctgatttacatcagtcacatgcactcagaccacctgagttaccccacactgaaggagctggctgggagaagaccggatattcccatttatgttggaaacacggaaagacctgtattttggaatctgaatcagagcggtgtccagttgaccaatatcaatatagtgccattcggaatatggcagcaggtagacaaaaatcttcgattcatgatcttgatggatggcgttcatcctgagatggacacttgcattattgtggagtataaaggtcataagatacttaatacagtggactgcaccagacccaatgggggaaggttgcctgagaaggttgctctaatgatgagtgattttgctggaggagcatcaggctttccaatgactttcagtggtggaaaatttaccgaggaatggaaagcccaattcattaaagcagagaggaagaagctcttgaactacaaggcccggctggtgaaggacctacaaccccgaatttattgcccctttgctgggtattttgtggaatctcacccatcagacaagtatattaaggaaacaaacatcaaaaatgacccaaatgaactcaataatcttatcaagaaaaactctgatgtggtaacgtggaccccacggcctggagccactcttgatctgagtcggatgctaaaggacccgacagacagcaagggcatcatagarcctccagaggggaccaagatctacaaggattcctgggactttgaaccctatttgaacatcttgaatgctgctgtaggagatgagatatttcttcactcatcctggataaaagaatacttcacytgggcyggatttaaggattacaacctggtggtcaggatgattgaaacagatgaggacttcagcccttttcctggaggatatgactatttggttgactttctagacttatcctttccaaaagagagaccaagccgggaacacccgtatgaggaaattcggagccgggttgacgtcatcagacacgtggtaaagaacggtcttctctgggacgacttgtatataggattccaaacccggctgcaacggagtcctgacatataccatcacctgttttggaaccattttcaaataaaactccctctcacgccacccaactggaggtccttcctgatgcactgtgggtagagcagacctgagctttccagagatgccaaacaacatagaaaattcaagaatttactgatgctacgtcttgaacacaggaagcttmtaccaaagggacttatgccttattgaaatcaacagtggataattacatgttgcatttgtgagaygttcacatatgtttgtggatcactacatagccagataatttagatttcacttattccatacacaattctctgtaaaagaggtgatgaaccctacaggaacagattgtctatgggaaaccaatcataacaggaagagatgtgaatctgagggttgaagaaatagracaggaggagacagaattccctcgtggaygacgaggaaactggaagggggtgaggtaacaaaagttgggttagaaaaaaaaaaaaaaaaaaaaaaaa

SEQ ID NO: 2 - protein, 578 aa, Felis catus
  Cytidin-Monophosphat-N-Acetylneuraminsäure-Hydroxylase (CMAH), CMAH-A Allel
MEQSIEQTTEVLLCLSPGEAADLKEGINFLRNKKTGKDFILYKSKNRVRACKNVCKHQGGLFIKDIEDLDGRSVRCTKHNWRLDVSTMKYVNPPGSFCQDELVVEMDEENGLLLLELNPPNPWDSEPRSPEHLAFGEVQITYLTHACMDLKLGDKRMVFDPWLTGPAFARGWWLLHEPPSDWLERLCQADLIYISHMHSDHLSYPTLKELAGRRPDIPIYVGNTERPVFWNLNQSGVQLTNINIVPFGIWQQVDKNLRFMILMDGVHPEMDTCIIVEYKGHKILNTVDCTRPNGGRLPEKVALMMSDFAGGASGFPMTFSGGKFTEEWKAQFIKAERKKLLNYKARLVKDLQPRIYCPFAGYFVESHPSDKYIKETNIKNDPNELNNLIKKNSDVVTWTPRPGATLDLSRMLKDPTDSKGIIEPPEGTKIYKDSWDFEPYLNILNAAVGDEIFLHSSWIKEYFTWAGFKDYNLVVRMIETDEDFSPFPGGYDYLVDFLDLSFPKERPSREHPYEEIRSRVDVIRHVVKNGLLWDDLYIGFQTRLQRSPDIYHHLFWNHFQIKLPLTPPNWRSFLMHCG

SEQ ID NO: 3 - DNA, 38 bp, Artificial Sequence
  Exon 1 Forward
tgtaaaacgacggccagttgagcaagcagagcgtgcat

SEQ ID NO: 4 - DNA, 42 bp, Artificial Sequence
  Exon 1 Reverse
gcaggaaacagctatgacaagtgagcacacacgaagattatg

SEQ ID NO: 5 - DNA, 45 bp, Artificial Sequence
  Exon 2 Forward
tgtaaaacgacggccagttgaagtggtgctcaagcccctcattta

SEQ ID NO: 6 - DNA, 43 bp, Artificial Sequence
  Exon 2 Reverse
gcaggaaacagctatgacctggtcacagtcttgtcctaggcac

SEQ ID NO: 7 - DNA, 48 bp, Artificial Sequence
  Exon 3 Forward
tgtaaaacgacggccagttgaccctttgatttttggtactctgtgtac

SEQ ID NO: 8 - DNA, 45 bp, Artificial Sequence
  Exon 3 Reverse
gcaggaaacagctatgacctaatacacacacataaatggacatct

SEQ ID NO: 9 - DNA, 46 bp, Artificial Sequence
  Exon 4 Forward
tgtaaaacgacggccagttgataaaaccaaccgggagagtttctat

SEQ ID NO: 10 - DNA, 45 bp, Artificial Sequence
  Exon 4 Reverse
gcaggaaacagctatgaccacacatgaaaactgtatgatattcgc

SEQ ID NO: 11 - DNA, 48 bp, Artificial Sequence
  Exon 5-6 Forward
tgtaaaacgacggccagttgaggagcaaactgtctcttctactaggtg

SEQ ID NO: 12 - DNA, 45 bp, Artificial Sequence
  Exon 5-6 Reverse
gcaggaaacagctatgaccgaaatgaagatagtagaagatggtta

SEQ ID NO: 13 - DNA, 48 bp, Artificial Sequence
  Exon 7 Forward
tgtaaaacgacggccagttgattccttggatagaagtaattcttctct

SEQ ID NO: 14 - DNA, 45 bp, Artificial Sequence
  Exon 7 Reverse
gcaggaaacagctatgaccgtttcccagttaagactgtaaacttc

SEQ ID NO: 15 - DNA, 47 bp, Artificial Sequence
  Exon 8 Forward
tgtaaaacgacggccagttgaagagagcactttctactcatgacaca

SEQ ID NO: 16 - DNA, 45 bp, Artificial Sequence
  Exon 8 Reverse
gcaggaaacagctatgaccagacaatctctctgaatggattctag

SEQ ID NO: 17 - DNA, 48 bp, Artificial Sequence
  Exon 9 Forward
tgtaaaacgacggccagttgaaagacaaagtataagtacaacttcttg

SEQ ID NO: 18 - DNA, 45 bp, Artificial Sequence
  Exon 9 Reverse
gcaggaaacagctatgaccacaaagacttaatattcctacaaacg

SEQ ID NO: 19 - DNA, 47 bp, Artificial Sequence
  Exon 10 Forward
tgtaaaacgacggccagttgacaaaagatgtggagttttcccatagt

SEQ ID NO: 20 - DNA, 42 bp, Artificial Sequence
  Exon 10 Reverse
gcaggaaacagctatgaccaacaatcgtgggacaagaatgct

SEQ ID NO: 21 - DNA, 49 bp, Artificial Sequence
  Exon 11 Forward
tgtaaaacgacggccagttgagagggactataccgaactccaattcatt

SEQ ID NO: 22 - DNA, 45 bp, Artificial Sequence
  Exon 11 Reverse
gcaggaaacagctatgaccgacaactagcacagtaaaggaaggtg

SEQ ID NO: 23 - DNA, 46 bp, Artificial Sequence
  Exon 12 Forward
tgtaaaacgacggccagttgatgcgttctgtagatgaggagactgc

SEQ ID NO: 24 - DNA, 44 bp, Artificial Sequence
  Exon 12 Reverse
gcaggaaacagctatgaccgaatgaagctctaatggtggaatct

SEQ ID NO: 25 - DNA, 44 bp, Artificial Sequence
  Exon 13 Forward
tgtaaaacgacggccagttgaaaatgccaggcactgaaacagta

SEQ ID NO: 26 - DNA, 44 bp, Artificial Sequence
  Exon 13 Reverse
gcaggaaacagctatgaccgatttagctctgaacactcactgcc

SEQ ID NO: 27 - DNA, 33 bp, Artificial Sequence
  Exon 14/15 3´-UTR Forward
tgtaaaacgacggccagttgacgtatagttcag

SEQ ID NO: 28 - DNA, 30 bp, Artificial Sequence
  Exon 14/15 3´-UTR Reverse
gcaggaaacagctatgacccctgactctct

SEQ ID NO: 29 - DNA, 30 bp, Artificial Sequence
  Exon 1a Forward
tgtaaaacgacggccagttgaaatttacag

SEQ ID NO: 30 - DNA, 30 bp, Artificial Sequence
  Exon 1a Reverse
gcaggaaacagctatgacctagcaaacata

SEQ ID NO: 31 - DNA, 42 bp, Artificial Sequence
  5´-UTR Forward
tgtaaaacgacggccagttgacgctctccttgctcagtgttg

SEQ ID NO: 32 - DNA, 30 bp, Artificial Sequence
  5´-UTR Reverse
gcaggaaacagctatgacccaacactgagc

SEQ ID NO: 33 - DNA, 21 bp, Artificial Sequence
  Forward-Primer T268A-BG5F (Genotyping-Assay 268)
cacaaagcacaactggaggtt

SEQ ID NO: 34 - DNA, 25 bp, Artificial Sequence
  Reverse-Primer T268A-BG5R (Genotyping-Assay 268)
caactagttcgtcttgacagaagct

SEQ ID NO: 35 - DNA, 19 bp, Artificial Sequence
  Reporter-Sonde T268A-BG5V1 (VIC-markiert)
caccatgaaatacgtcaat

SEQ ID NO: 36 - DNA, 18 bp, Artificial Sequence
  Reporter-Sonde T268A-BG5M1 (FAM-markiert)
accatgaaaaacgtcaat

SEQ ID NO: 37 - DNA, 28 bp, Artificial Sequence
  Forward-Primer G142A-BG4F (Genotyping-Assay)
gcaaagatttcattctgtacaagagcaa

SEQ ID NO: 38 - DNA, 22 bp, Artificial Sequence
  Reverse-Primer G142A-BG4R (Genotyping-Assay)
cttgatgcttgcacacgttctt

SEQ ID NO: 39 - DNA, 14 bp, Artificial Sequence
  Reporter-Sonde G142A-BG4V2 (VIC)
ccctcacgcgattc

SEQ ID NO: 40 - DNA, 14 bp, Artificial Sequence
  Reporter-Sonde G142A-BG4M2 (FAM)
ccctcatgcgattc

SEQ ID NO: 41 - DNA, 22 bp, Artificial Sequence
  Forward-Primer CMAH_F (Genotyping-Assay)
ggtgcaacggaatcagtagtga

SEQ ID NO: 42 - DNA, 20 bp, Artificial Sequence
  Reverse-Primer CMAH_R (Genotyping-Assay)
gcctctccctgggaattctg

SEQ ID NO: 43 - DNA, 23 bp, Artificial Sequence
  Reporter-Sonde CMAH_wt (YAK-BBQ)
cagcttcggttgctcgtttgctc

SEQ ID NO: 44 - DNA, 22 bp, Artificial Sequence
  Reporter-Sonde CMAH_mut (FAM-BBQ)
acggtggttgctcgtttgctcc